European Patent Application EP 4 711 379 A1, published March 18, 2026. Title: Method for Producing botulinum neurotoxin using soluble partner and GP41.1 intein. Applicant: MVRIX Co., Ltd. Application EP EP25156613.9, filed February 7, 2025. The sequence listing filed with the application follows.

SEQUENCE LISTING (18 sequences)

SEQ ID NO: 1 - DNA, 717 bp, synthetic construct
  source 1..717: mol_type = other DNA
atggtgagcaagggcgaggagctgttcaccggggtggtgcccatcctggtcgagctggacggcgacgtaaacggccacaagttcagcgtgtccggcgagggcgagggcgatgccacctacggcaagctgaccctgaagttcatctgcaccaccggcaagctgcccgtgccctggcccaccctcgtgaccaccctgacctacggcgtgcagtgcttcagccgctaccccgaccacatgaagcagcacgacttcttcaagtccgccatgcccgaaggctacgtccaggagcgcaccatcttcttcaaggacgacggcaactacaagacccgcgccgaggtgaagttcgagggcgacaccctggtgaaccgcatcgagctgaagggcatcgacttcaaggaggacggcaacatcctggggcacaagctggagtacaactacaacagccacaacgtctatatcatggccgacaagcagaagaacggcatcaaggtgaacttcaagatccgccacaacatcgaggacggcagcgtgcagctcgccgaccactaccagcagaacacccccatcggcgacggccccgtgctgctgcccgacaaccactacctgagcacccagtccgccctgagcaaagaccccaacgagaagcgcgatcacatggtcctgctggagttcgtgaccgccgccgggatcactctcggcatggacgagctgtacaag

SEQ ID NO: 2 - DNA, 294 bp, synthetic construct
  source 1..294: mol_type = other DNA
atgtcggactcagaagtcaatcaagaagctaagccagaggtcaagccagaagtcaagcctgagactcacatcaatttaaaggtgtccgatggatcttcagagatcttcttcaagatcaaaaagaccactcctttaagaaggctgatggaagcgttcgctaaaagacagggtaaggaaatggactccttaagattcttgtacgacggtattagaattcaagctgatcagacccctgaagatttggacatggaggataacgatattattgaggctcacagagaacagattggtggt

SEQ ID NO: 3 - DNA, 1113 bp, synthetic construct
  source 1..1113: mol_type = other DNA
atgaaaatcgaagaaggtaaactggtaatctggattaacggcgataaaggctataacggtctcgctgaagtcggtaagaaattcgagaaagataccggaattaaagtcaccgttgagcatccggataaactggaagagaaattcccacaggttgcggcaactggcgatggccctgacattatcttctgggcacacgaccgctttggtggctacgctcaatctggcctgttggctgaaatcaccccggacaaagcgttccaggacaagctgtatccgtttacctgggatgccgtacgttacaacggcaagctgattgcttacccgatcgctgttgaagcgttatcgctgatttataacaaagatctgctgccgaacccgccaaaaacctgggaagagatcccggcgctggataaagaactgaaagcgaaaggtaagagcgcgctgatgttcaacctgcaagaaccgtacttcacctggccgctgattgctgctgacgggggttatgcgttcaagtatgaaaacggcaagtacgacattaaagacgtgggcgtggataacgctggcgcgaaagcgggtctgaccttcctggttgacctgattaaaaacaaacacatgaatgcagacaccgattactccatcgcagaagctgcctttaataaaggcgaaacagcgatgaccatcaacggcccgtgggcatggtccaacatcgacaccagcaaagtgaattatggtgtaacggtactgccgaccttcaagggtcaaccatccaaaccgttcgttggcgtgctgagcgcaggtattaacgccgccagtccgaacaaagagctggcaaaagagttcctcgaaaactatctgctgactgatgaaggtctggaagcggttaataaagacaaaccgctgggtgccgtagcgctgaagtcttacgaggaagagttggcgaaagatccacgtattgccgccactatggaaaacgcccagaaaggtgaaatcatgccgaacatcccgcagatgtccgctttctggtatgccgtgcgtactgcggtgatcaacgccgccagcggtcgtcagactgtcgatgaagccctgaaagacgcgcagactaattcgagctcg

SEQ ID NO: 4 - DNA, 30 bp, synthetic construct
  source 1..30: mol_type = other DNA
cgtcgccggcgtcgccggagacgtcgccgt

SEQ ID NO: 5 - DNA, 120 bp, synthetic construct
  source 1..120: mol_type = other DNA
atgatgctgaaaaaaatcctgaaaatcgaggaactggatgaacgcgaactgattgatattgaagttagcggtaaccacctgttctatgccaatgatattctgacccataatagcagcagc

SEQ ID NO: 6 - DNA, 273 bp, synthetic construct
  source 1..273: mol_type = other DNA
agtggttattgcctggatctgaaaacccaggttcagacaccgcagggtatgaaagaaatttcaaatattcaggtgggtgatctggttctgagcaataccggttataatgaagtgctgaatgtgttcccgaaaagcaagaaaaaaagctacaaaatcaccctggaagatggcaaagaaattatctgtagcgaagaacacctgtttccgacacagaccggtgaaatgaatattagcggtggtctgaaagaaggtatgtgcctgtatgttaaagaa

SEQ ID NO: 7 - DNA, 402 bp, synthetic construct
  source 1..402: mol_type = other DNA
gaagcgcgcgattgggtgaaacgcgtgggcggcaaaaccagcctgagcgtgaacacctatagcggcgaagtggaacgcaaaaacattaactatattatgaaacataccgtgaaaaaacgcatgtttaaaattaaagcgggcggcaaagaagtgattgtgaccgcggatcatagcgtgatggtgaaacgcgatggcaaaattattgatgtgaaaccgaccgaaatgaaacagaccgatcgcgtggtgaaatggatgctgaccggcagccatatgattgaatttattgaatttgaaattgaagatctgggcgtgatggaaattgatgtgtatgatattgaagtggatggcaaccataacttttttggcaacgatattctggtgcataacagcgtgtatctgaac

SEQ ID NO: 8 - DNA, 93 bp, synthetic construct
  source 1..93: mol_type = other DNA
tatattgataccgatagcgtggtgggcgataccattattgatgtgagcggcaaaaaaatgaccattgcggaattttatgatagcaccccggat

SEQ ID NO: 9 - DNA, 519 bp, synthetic construct
  source 1..519: mol_type = other DNA
atgcaggaagcgaaaattgatattaaaagcctgtatgatagcctggcgaaaaaatatgatgtgcagcataaaaacagctatgaagtgatttatccgaaaggctatgaaattaaagtgctgggcaacaaatatgtgaaactggtggcgatgagccgccataaaacccagaaacatctggtgaaaattgtggtgaaaagcgaaaaaaccattgatagcctggatccgattcgccagaaaagcctgctgaaaaaacaggatgaagtggtggtgaccaccgatcatattgcgatggtgtatcgcgatgatcatttttttgaaaacgtgaacgcgaaaaacctgaaagtgggcaactatgtgagcgtgtatgatgaagcgagcgataaagaagtgattggcgaaattgcgagcattgaagatctgggcatgaccgatgattatgtgtatgatgcggaagtggatgatgatagccatgcgttttatgcgagcaacattctggtgcataacagccagtttgcgaac

SEQ ID NO: 10 - DNA, 60 bp, synthetic construct
  source 1..60: mol_type = other DNA
agcggcgataccgatagcgtgcatggcaaaacccatgtgtttattcgcagcattaaaaac

SEQ ID NO: 11 - DNA, 1314 bp, synthetic construct
  source 1..1314: mol_type = other DNA
atgccgtttgtgaacaaacagttcaactataaagatccggtgaacggtgttgatatcgcctatatcaaaattccgaatgcaggtcagatgcagccggttaaagcctttaaaatccataacaaaatttgggtgattccggaacgtgatacctttaccaatccggaagaaggtgatctgaatccgcctccggaagcaaaacaggttccggttagctattatgatagcacctatctgagcaccgataacgagaaagataactatctgaaaggtgtgaccaaactgtttgaacgcatttatagtaccgatctgggtcgtatgctgctgaccagcattgttcgtggtattccgttttggggtggtagcaccattgataccgaactgaaagttattgacaccaactgcattaatgtgattcagccggatggtagctatcgtagcgaagaactgaatctggttattattggtccgagcgcagatatcattcagtttgaatgtaaaagctttggccacgatgttctgaatctgacccgtaatggttatggtagtacccagtatattcgtttcagtccggattttacctttggctttgaagaaagcctggaagttgatacaaatccgctgttaggtgcaggtaaatttgcaaccgatccggcagttaccctggcacatgaactgattcatgccgaacatcgtctgtatggtattgccattaatccgaatcgtgtgttcaaagtgaataccaacgcctattatgaaatgagcggtctggaagtgagttttgaagaactgcgtacctttggtggtcatgatgccaaatttatcgatagcctgcaagaaaatgaatttcgcctgtactactataacaaattcaaagatgttgcgagcaccctgaataaagccaaaagcattattggcaccaccgcaagcctgcagtatatgaaaaatgtgtttaaagaaaaatatctgctgagcgaagataccagcggtaaatttagcgttgacaaactgaaattcgataaactgtacaagatgctgaccgagatttataccgaagataacttcgtgaacttctttaaggtgatcaaccgcaaaacctacctgaactttgataaagccgtgtttcgcattaacattgtgccggatgaaaactacaccatcaaagatggctttaatctgaagggtgcaaatctgtccaccaattttaacggtcagaacaccgaaattaacagccgtaattttacccgtctgaaaaactttaccggtctgttcgaattttacaaactgctgtgtgttcgtggcattatcccgtttaaa

SEQ ID NO: 12 - DNA, 1272 bp, synthetic construct
  source 1..1272: mol_type = other DNA
gcactgaatgatctgtgcatcaaagtgaataattgggacctgttttttagcccgagcgaagataactttaccaacgatctggataaagtggaagaaattaccgcagataccaatattgaagcagccgaagaaaacattagcctggatctgattcagcagtattatctgaccttcgattttgataacgagccggaaaatatcagcattgaaaatctgagcagcgatattattggtcagctggaaccgatgccgaatattgaacgttttccgaatggcaaaaaatacgagctggacaaatataccatgttccattatctgcgtgcccaagaatttgaacatggtgatagccgcattattctgaccaattcagcagaagaagcactgctgaaaccgaatgttgcatatacctttttcagcagcaaatatgtgaaaaaaatcaacaaagccgtcgaagcctttatgtttctgaattgggctgaagaactggtgtatgatttcaccgatgaaaccaatgaagttaccaccatggataaaattgccgacattaccattatcgtgccgtatattggtccggctctaaatattggcaatatgctgagcaaaggtgaatttgtggaagccattatctttaccggtgttgttgcaatgctggaatttatcccggaatatgcactgccggtttttggcacctttgcaattgttagctatatcgccaataaagttctgaccgttcagaccattaataacgcactgagcaaacgcaatgagaaatgggatgaagtgtataaatacaccgttaccaattggctggccaaagttaatacccagattgatctgatccgcgagaaaatgaaaaaagccctggaaaatcaggcagaagcaaccaaagcaattatcaactatcagtacaaccagtacaccgaggaagagaaaaacaacatcaacttcaacatcgatgacctgagcagcaaactgaatgaaagcattaatagcgccatgattaacatcaacaagtttctggatcagtgcagcgttagctatctgatgaatagcatgattccgtatgcagtgaaacgcctgaaagattttgatgcaagcgttcgtgatgtcctgctgaaatatatctatgataatcgtggcaccctggttctgcaggttgatcgtctgaaagatgaagttaataacaccctgagcgcagatattccgtttcagctgagtaaatatgtggacaacaaaaaactgctgagcacctttaccgagtacatcaaaaac

SEQ ID NO: 13 - DNA, 1272 bp, synthetic construct
  source 1..1272: mol_type = other DNA
attgtgaacaccagcattctgagcatcgtgtacaaaaaagatgatctgattgatctgagccgctatggtgccaaaatcaatattggtgatcgcgtgtattatgatagcatcgacaaaaaccagatcaaactgattaatctggaaagcagcaccattgaggtgattctgaaaaatgccattgtgtataacagcatgtacgagaatttttcgaccagcttctggattaaaatccccaaatacttcagcaaaatcaacctgaacaacgagtacaccattatcaactgcattgaaaacaatagcggttggaaagtgagcctgaattatggtgaaattatctggaccctgcaggacaacaaacagaatattcagcgtgtggtgttcaaatatagccagatggtgaatatcagcgattacattaaccgctggatttttgtgaccattaccaataatcgtctgaccaagagcaagatctatattaacggtcgtctgattgaccagaaaccgattagcaatctgggtaatattcatgccagcaacaagatcatgtttaaactggatggttgtcgtgatccgcgtcgctatattatgatcaaatactttaacctgtttgacaaagaactgaacgaaaaagaaatcaaagacctgtatgatagccagagcaatagcggcattctgaaagatttttggggtaactatctgcagtatgacaaaccgtattatatgctgaacctgttcgatccgaacaaatatgtggatgtgaacaatattggcatccgtggctatatgtatctgaaaggtccgcgtggtagcgttgttaccaccaacatttatctgaatagcaccctgtatgaaggcaccaaattcatcattaaaaagtatgccagcggcaacgaagataatattgtgcgtaataatgaccgcgtgtatatcaatgttgtggtgaagaataaagaatatcgcctggcaaccaatgcaagccaggcaggcgttgaaaaaattctgagcgcactggaaattccggatgttggtaatctgagccaggttgttgttatgaaaagcaaagatgaccagggcattcgcaacaaatgcaaaatgaatctgcaggataataacggcaacgatattggctttatcggcttccatctgtatgacaatattgcaaaactggttgcgagcaattggtataatcgtcaggttggtaaagcaagccgtacctttggttgtagctgggaatttattccggttgatgatggttggggtgaaagcagcctg

SEQ ID NO: 14 - DNA, 18 bp, synthetic construct
  source 1..18: mol_type = other DNA
ctggttccgcgtggtagc

SEQ ID NO: 15 - DNA, 18 bp, synthetic construct
  source 1..18: mol_type = other DNA
catcatcatcaccaccac

SEQ ID NO: 16 - protein, 6 aa, synthetic construct
SGYSSS

SEQ ID NO: 17 - protein, 10 aa, synthetic construct
YIDTDSVYLN

SEQ ID NO: 18 - protein, 6 aa, synthetic construct
SGDTDS